European Patent Application EP 4 144 371 A1, published March 8, 2023. Title: COMBINATION DRUG FOR TREATING KIDNEY CANCER. Applicant: CHIA TAI TIANQING PHARMACEUTICAL GROUP CO., LTD. The sequence listing filed with the application follows.

SEQUENCE LISTING (21 sequences)

SEQ ID NO: 1 - protein, 5 aa, Mus sp.
TYGVH

SEQ ID NO: 2 - protein, 16 aa, Mus sp.
VIWRGVTTDYNAAFMS

SEQ ID NO: 3 - protein, 8 aa, Mus sp.
LGFYAMDY

SEQ ID NO: 4 - protein, 5 aa, Mus sp.
SYGMS

SEQ ID NO: 5 - protein, 16 aa, Mus sp.
SISSGGSTYYPDSVKG

SEQ ID NO: 6 - protein, 8 aa, Mus sp.
GYDSGFAY

SEQ ID NO: 7 - protein, 11 aa, Mus sp.
KASQSVSNDVA

SEQ ID NO: 8 - protein, 7 aa, Mus sp.
YAANRYT

SEQ ID NO: 9 - protein, 9 aa, Mus sp.
QQDYTSPYT

SEQ ID NO: 10 - protein, 14 aa, Mus sp.
ASQSVSTSSSSFMH

SEQ ID NO: 11 - protein, 7 aa, Mus sp.
YASNLES

SEQ ID NO: 12 - protein, 9 aa, Mus sp.
QHSWEIPYT

SEQ ID NO: 13 - protein, 116 aa, Artificial Sequence
  heavy chain variable region of hu5G11-hIgG1 and hu5G11-hIgG4
QITLKESGPTLVKPTQTLTLTCTVSGFSLSTYGVHWIRQPPGKALEWLGVIWRGVTTDYNAAFMSRLTITKDNSKNQVVLTMNNMDPVDTATYYCARLGFYAMDYWGQGTLVTVSS

SEQ ID NO: 14 - protein, 116 aa, Artificial Sequence
  heavy chain variable region of hu13C5-hIgG1 and hu13C5-hIgG4
EVQLVESGGGLVKPGGSLRLSCAASGFIFRSYGMSWVRQAPGKGLEWVASISSGGSTYYPDSVKGRFTISRDNAKNSLYLQMNSLRAEDTAVYDCARGYDSGFAYWGQGTLVTVSS

SEQ ID NO: 15 - protein, 107 aa, Artificial Sequence
  light chain variable region of hu5G11-hIgG1 and hu5G11-hIgG4
DIQMTQSPSSLSASVGDRVTITCKASQSVSNDVAWYQQKPGKAPKLLIYYAANRYTGVPDRFSGSGYGTDFTFTISSLQPEDIATYFCQQDYTSPYTFGQGTKLEIK

SEQ ID NO: 16 - protein, 111 aa, Artificial Sequence
  light chain variable region of hu13C5-hIgG1 and hu13C5-hIgG4
DIVLTQSPASLAVSPGQRATITCRASQSVSTSSSSFMHWYQQKPGQPPKLLIKYASNLESGVPARFSGSGSGTDFTLTINPVEANDTANYYCQHSWEIPYTFGQGTKLEIK

SEQ ID NO: 17 - protein, 446 aa, Artificial Sequence
  heavy chain of h5G11-hIgG1
QITLKESGPTLVKPTQTLTLTCTVSGFSLSTYGVHWIRQPPGKALEWLGVIWRGVTTDYNAAFMSRLTITKDNSKNQVVLTMNNMDPVDTATYYCARLGFYAMDYWGQGTLVTVSSASTKGPSVFPLAPSSKSTSGGTAALGCLVKDYFPEPVTVSWNSGALTSGVHTFPAVLQSSGLYSLSSVVTVPSSSLGTQTYICNVNHKPSNTKVDKKVEPKSCDKTHTCPPCPAPELLGGPSVFLFPPKPKDTLMISRTPEVTCVVVAVSHEDPEVKFNWYVDGVEVHNAKTKPREEQYNSTYRVVSVLTVLHQDWLNGKEYKCKVSNKALPAPIEKTISKAKGQPREPQVYTLPPSRDELTKNQVSLTCLVKGFYPSDIAVEWESNGQPENNYKTTPPVLDSDGSFFLYSKLTVDKSRWQQGNVFSCSVMHEALHNHYTQKSLSLSPGK

SEQ ID NO: 18 - protein, 214 aa, Artificial Sequence
  light chain of h5G11-hIgG1 and h5G11-hIgG4
DIQMTQSPSSLSASVGDRVTITCKASQSVSNDVAWYQQKPGKAPKLLIYYAANRYTGVPDRFSGSGYGTDFTFTISSLQPEDIATYFCQQDYTSPYTFGQGTKLEIKRTVAAPSVFIFPPSDEQLKSGTASVVCLLNNFYPREAKVQWKVDNALQSGNSQESVTEQDSKDSTYSLSSTLTLSKADYEKHKVYACEVTHQGLSSPVTKSFNRGEC

SEQ ID NO: 19 - protein, 446 aa, Artificial Sequence
  heavy chain of hu13C5-hIgG1
EVQLVESGGGLVKPGGSLRLSCAASGFIFRSYGMSWVRQAPGKGLEWVASISSGGSTYYPDSVKGRFTISRDNAKNSLYLQMNSLRAEDTAVYDCARGYDSGFAYWGQGTLVTVSSASTKGPSVFPLAPSSKSTSGGTAALGCLVKDYFPEPVTVSWNSGALTSGVHTFPAVLQSSGLYSLSSVVTVPSSSLGTQTYICNVNHKPSNTKVDKKVEPKSCDKTHTCPPCPAPELLGGPSVFLFPPKPKDTLMISRTPEVTCVVVAVSHEDPEVKFNWYVDGVEVHNAKTKPREEQYNSTYRVVSVLTVLHQDWLNGKEYKCKVSNKALPAPIEKTISKAKGQPREPQVYTLPPSRDELTKNQVSLTCLVKGFYPSDIAVEWESNGQPENNYKTTPPVLDSDGSFFLYSKLTVDKSRWQQGNVFSCSVMHEALHNHYTQKSLSLSPGK

SEQ ID NO: 20 - protein, 218 aa, Artificial Sequence
  light chain of hu13C5-hIgG1 and hu13C5-hIgG4
DIVLTQSPASLAVSPGQRATITCRASQSVSTSSSSFMHWYQQKPGQPPKLLIKYASNLESGVPARFSGSGSGTDFTLTINPVEANDTANYYCQHSWEIPYTFGQGTKLEIKRTVAAPSVFIFPPSDEQLKSGTASVVCLLNNFYPREAKVQWKVDNALQSGNSQESVTEQDSKDSTYSLSSTLTLSKADYEKHKVYACEVTHQGLSSPVTKSFNRGEC

SEQ ID NO: 21 - protein, 442 aa, Artificial Sequence
  heavy chain of hu5G11-hIgG4
QITLKESGPTLVKPTQTLTLTCTVSGFSLSTYGVHWIRQPPGKALEWLGVIWRGVTTDYNAAFMSRLTITKDNSKNQVVLTMNNMDPVDTATYYCARLGFYAMDYWGQGTLVTVSSASTKGPSVFPLAPCSRSTSESTAALGCLVKDYFPEPVTVSWNSGALTSGVHTFPAVLQSSGLYSLSSVVTVPSSSLGTKTYTCNVDHKPSNTKVDKRVESKYGPPCPPCPAPEAAGGPSVFLFPPKPKDTLMISRTPEVTCVVVDVSQEDPEVQFNWYVDGVEVHNAKTKPREEQFNSTYRVVSVLTVLHQDWLNGKEYKCKVSNKGLPSSIEKTISKAKGQPREPQVYTLPPSQEEMTKNQVSLTCLVKGFYPSDIAVEWESNGQPENNYKTTPPVLDSDGSFFLYSRLTVDKSRWQEGNVFSCSVMHEALHNHYTQKSLSLSLG